European Patent Application EP 4 458 973 A1, published November 6, 2024. Title: 면역 회피성 항종양 아데노바이러스. Applicant: (주)큐리진. Application KR. The sequence listing filed with the application follows.

SEQUENCE LISTING (20 sequences)

SEQ ID NO: 1 - DNA, 87 bp, synthetic construct
  source 1..87: mol_type = other DNA
atgctgaccaaggcggtttttgatgcaaataaaaaacaggcgggttctttgcccggtaacggcaaatacgcgggcaaccacaaatac

SEQ ID NO: 2 - protein, 29 aa, synthetic construct
MLTKAVFDANKKQAGSLPGNGKYAGNHKY

SEQ ID NO: 3 - DNA, 165 bp, synthetic construct
  source 1..165: mol_type = other DNA
atggatatgacggttccggcattcctgaccaaggcggtttttgatgcaaataaaaaacaggcgggttctttgcccggtaacggcaaatacgcgggcaaccacaaatacggcggactgtttaccaacggcgaaaacggtgcgctggtgggcgcggaatacggtacg

SEQ ID NO: 4 - protein, 55 aa, synthetic construct
MDMTVPAFLTKAVFDANKKQAGSLPGNGKYAGNHKYGGLFTNGENGALVGAEYGT

SEQ ID NO: 5 - protein, 15 aa, synthetic construct
GGGGSGGGGSGGGGS

SEQ ID NO: 6 - DNA, 129 bp, synthetic construct
  source 1..129: mol_type = other DNA
ccaaatccttgcgaatgggatgaagctgctactgctcttgaaataaacctagaagaagaggacgatgacaacgaagacgaagtagacgagcaagctgagcagcaaaaaactcacgtatttgggcaggcg

SEQ ID NO: 7 - protein, 59 aa, synthetic construct
PNPCEWDEAATALEINLEEEDDDNEDEVDEQAEQQKTHVFGQAPYSGINITKEGIQIGV

SEQ ID NO: 8 - DNA, 216 bp, synthetic construct
  source 1..216: mol_type = other DNA
ccaaatccttgcgaatgggatgaagctgctactgctcttgaaataaacctagaagaagaggacgatgacaacgaaatgctgaccaaggcggtttttgatgcaaataaaaaacaggcgggttctttgcccggtaacggcaaatacgcgggcaaccacaaatacgacgaagtagacgagcaagctgagcagcaaaaaactcacgtatttgggcaggcg

SEQ ID NO: 9 - protein, 88 aa, synthetic construct
PNPCEWDEAATALEINLEEEDDDNEMLTKAVFDANKKQAGSLPGNGKYAGNHKYDEVDEQAEQQKTHVFGQAPYSGINITKEGIQIGV

SEQ ID NO: 10 - DNA, 384 bp, synthetic construct
  source 1..384: mol_type = other DNA
ccaaatccttgcgaatgggatgaagctgctactgctcttgaaataaacctagaagaagaggacgatgacaacgaaggtgggggtggcagtggtgggggtggtagtggaggaggagggtctatggatatgacggttccggcattcctgaccaaggcggtttttgatgcaaataaaaaacaggcgggttctttgcccggtaacggcaaatacgcgggcaaccacaaatacggcggactgtttaccaacggcgaaaacggtgcgctggtgggcgcggaatacggtacgggtgggggtggcagtggtgggggtggtagtggaggaggagggtctgacgaagtagacgagcaagctgagcagcaaaaaactcacgtatttgggcaggcg

SEQ ID NO: 11 - protein, 144 aa, synthetic construct
PNPCEWDEAATALEINLEEEDDDNEGGGGSGGGGSGGGGSMDMTVPAFLTKAVFDANKKQAGSLPGNGKYAGNHKYGGLFTNGENGALVGAEYGTGGGGSGGGGSGGGGSDEVDEQAEQQKTHVFGQAPYSGINITKEGIQIGV

SEQ ID NO: 12 - DNA, 327 bp, synthetic construct
  source 1..327: mol_type = other DNA
ccaaatccttgcgaatgggatgaagctgctactgctcttgaaataaacctagaagaagaggacgatgacaacgaaatgatgggctgtagcagccatgagcatgagcatgaggatgaagccgtcgacgcgaattcattagctgctgctaaagagacggctctgtatcatcttgacaggttgggagtagctgacgcttacaaggatctaatcgataaagccaaaactgttgaaggtgtaaaggcacggtattttgaaattttacatgcattacccgacgaagtagacgagcaagctgagcagcaaaaaactcacgtatttgggcaggcg

SEQ ID NO: 13 - protein, 124 aa, synthetic construct
PNPCEWDEAATALEINLEEEDDDNEMGCSSHEHEHEDEAVDANSLAAAKETALYHLDRLGVADAYKDLIDKAKTVEGVKARYFEILHALPDEVDEQAEQQKTHVFGQAPYSGINITKEGIQIGV

SEQ ID NO: 14 - DNA, 2859 bp, unidentified
  source 1..2859: mol_type = genomic DNA
atggctaccccttcgatgatgccgcagtggtcttacatgcacatctcgggccaggacgcctcggagtacctgagccccgggctggtgcagtttgcccgcgccaccgagacgtacttcagcctgaataacaagtttagaaaccccacggtggcgcctacgcacgacgtgaccacagaccggtcccagcgtttgacgctgcggttcatccctgtggaccgtgaggatactgcgtactcgtacaaggcgcggttcaccctagctgtgggtgataaccgtgtgctggacatggcttccacgtactttgacatccgcggcgtgctggacaggggccctacttttaagccctactctggcactgcctacaacgccctggctcccaagggtgccccaaatccttgcgaatgggatgaagctgctactgctcttgaaataaacctagaagaagaggacgatgacaacgaagacgaagtagacgagcaagctgagcagcaaaaaactcacgtatttgggcaggcgccttattctggtataaatattacaaaggagggtattcaaataggtgtcgaaggtcaaacacctaaatatgccgataaaacatttcaacctgaacctcaaataggagaatctcagtggtacgaaacagaaattaatcatgcagctgggagagtcctaaaaaagactaccccaatgaaaccatgttacggttcatatgcaaaacccacaaatgaaaatggagggcaaggcattcttgtaaagcaacaaaatggaaagctagaaagtcaagtggaaatgcaatttttctcaactactgaggcagccgcaggcaatggtgataacttgactcctaaagtggtattgtacagtgaagatgtagatatagaaaccccagacactcatatttcttacatgcccactattaaggaaggtaactcacgagaactaatgggccaacaatctatgcccaacaggcctaattacattgcttttagggacaattttattggtctaatgtattacaacagcacgggtaatatgggtgttctggcgggccaagcatcgcagttgaatgctgttgtagatttgcaagacagaaacacagagctttcataccagcttttgcttgattccattggtgatagaaccaggtacttttctatgtggaatcaggctgttgacagctatgatccagatgttagaattattgaaaatcatggaactgaagatgaacttccaaattactgctttccactgggaggtgtgattaatacagagactcttaccaaggtaaaacctaaaacaggtcaggaaaatggatgggaaaaagatgctacagaattttcagataaaaatgaaataagagttggaaataattttgccatggaaatcaatctaaatgccaacctgtggagaaatttcctgtactccaacatagcgctgtatttgcccgacaagctaaagtacagtccttccaacgtaaaaatttctgataacccaaacacctacgactacatgaacaagcgagtggtggctcccgggctagtggactgctacattaaccttggagcacgctggtcccttgactatatggacaacgtcaacccatttaaccaccaccgcaatgctggcctgcgctaccgctcaatgttgctgggcaatggtcgctatgtgcccttccacatccaggtgcctcagaagttctttgccattaaaaacctccttctcctgccgggctcatacacctacgagtggaacttcaggaaggatgttaacatggttctgcagagctccctaggaaatgacctaagggttgacggagccagcattaagtttgatagcatttgcctttacgccaccttcttccccatggcccacaacaccgcctccacgcttgaggccatgcttagaaacgacaccaacgaccagtcctttaacgactatctctccgccgccaacatgctctaccctatacccgccaacgctaccaacgtgcccatatccatcccctcccgcaactgggcggctttccgcggctgggccttcacgcgccttaagactaaggaaaccccatcactgggctcgggctacgacccttattacacctactctggctctataccctacctagatggaaccttttacctcaaccacacctttaagaaggtggccattacctttgactcttctgtcagctggcctggcaatgaccgcctgcttacccccaacgagtttgaaattaagcgctcagttgacggggagggttacaacgttgcccagtgtaacatgaccaaagactggttcctggtacaaatgctagctaactataacattggctaccagggcttctatatcccagagagctacaaggaccgcatgtactccttctttagaaacttccagcccatgagccgtcaggtggtggatgatactaaatacaaggactaccaacaggtgggcatcctacaccaacacaacaactctggatttgttggctaccttgcccccaccatgcgcgaaggacaggcctaccctgctaacttcccctatccgcttataggcaagaccgcagttgacagcattacccagaaaaagtttctttgcgatcgcaccctttggcgcatcccattctccagtaactttatgtccatgggcgcactcacagacctgggccaaaaccttctctacgccaactccgcccacgcgctagacatgacttttgaggtggatcccatggacgagcccacccttctttatgttttgtttgaagtctttgacgtggtccgtgtgcaccagccgcaccgcggcgtcatcgaaaccgtgtacctgcgcacgcccttctcggccggcaacgccacaacataa

SEQ ID NO: 15 - DNA, 3762 bp, synthetic construct
  source 1..3762: mol_type = other DNA
tggcccctccctcgggttaccccacagcctaggccgattcgacctctctccgctggggccctcgctggcgtccctgcaccctgggagcgcgagcggcgcgcgggcggggaagcgcggcccagacccccgggtccgcccggagcagctgcgctgtcggggccaggccgggctcccagtggattcgcgggcacagacgcccaggaccgcgctccccacgtggcggagggactggggacccgggcacccgtcctgccccttcaccttccagctccgcctcctccgcgcggaccccgccccgtcccgacccctcccgggtccccggcccagccccctccgggccctcccagcccctccccttcctttccgcggccccgccctctcctcgcggcgcgagtttcaggcagcgctgcgtcctgctgcgcacgtgggaagccctggccccggccacccccgcgactagtacaccgggactgaaaatgagacatattatctgccacggaggtgttattaccgaagaaatggccgccagtcttttggaccagctgatcgaagaggtactggctgataatcttccacctcctagccattttgaaccacctacccttcacgaactgtatgatttagacgtgacggcccccgaagatcccaacgaggaggcggtttcgcagatttttcccgactctgtaatgttggcggtgcaggaagggattgacttactcacttttccgccggcgcccggttctccggagccgcctcacctttcccggcagcccgagcagccggagcagagagccttgggtccggtttctatgccaaaccttgtaccggaggtgatcgatcttacctgccacgaggctggctttccacccagtgacgacgaggatgaagagggtgaggagtttgtgttagattatgtggagcaccccgggcacggttgcaggtcttgtcattatcaccggaggaatacgggggacccagatattatgtgttcgctttgctatatgaggacctgtggcatgtttgtctacagtcctgtgtctgaacctgagcctgagcccgagccagaaccggagcctgcaagacctacccgccgtcctaaaatggcgcctgctatcctgagacgcccgacatcacctgtgtctagagaatgcaatagtagtacggatagctgtgactccggtccttctaacacacctcctgagatacacccggtggtcccgctgtgccccattaaaccagttgccgtgagagttggtgggcgtcgccaggctgtggaatgtatcgaggacttgcttaacgagcctgggcaacctttggacttgagctgtaaacgccccaggccataaggtgtaaacctgtgacccctctccctcccccccctaacgttactggccgaagccgcttggaataaggccggtgtgcgtttgtctatatgttattttccaccatattgccgtcttttggcaatgtgagggcccggaaacctggccctgtcttcttgacgagcattcctaggggtctttcccctctcgccaaaggaatgcaaggtctgttgaatgtcgtgaaggaagcagttcctctggaagcttcttgaagacaaacaacgtctgtagcgaccctttgcaggcagcggaaccccccacctggcgacaggtgcctctgcggccaaaagccacgtgtataagatacacctgcaaaggcggcacaaccccagtgccacgttgtgagttggatagttgtggaaagagtcaaatggctctcctcaagcgtattcaacaaggggctgaaggatgcccagaaggtaccccattgtatgggatctgatctggggcctcggtgcacatgctttacatgtgtttagtcgaggttaaaaaaacgtctaggccccccgaaccacggggacgtggttttcctttgaaaaacacgatgataagcttgccacaacccgggatcctctagagtcgacatggaggcttgggagtgtttggaagatttttctgctgtgcgtaacttgctggaacagagctctaacagtacctcttggttttggaggtttctgtggggctcatcccaggcaaagttagtctgcagaattaaggaggattacaagtgggaatttgaagagcttttgaaatcctgtggtgagctgtttgattctttgaatctgggtcaccaggcgcttttccaagagaaggtcatcaagactttggatttttccacaccggggcgcgctgcggctgctgttgcttttttgagttttataaaggataaatggagcgaagaaacccatctgagcggggggtacctgctggattttctggccatgcatctgtggagagcggttgtgagacacaagaatcgcctgctactgttgtcttccgtccgcccggcgataataccgacggaggagcagcagcagcagcaggaggaagccaggcggcggcggcaggagcagagcccatggaacccgagagccggcctggaccctcgggaatgaatgttgtacaggtggctgaactgtatccagaactgagacgcattttgacaattacagaggatgggcaggggctaaagggggtaaagagggagcggggggcttgtgaggctacagaggaggctaggaatctagcttttagcttaatgaccagacaccgtcctgagtgtattacttttcaacagatcaaggataattgcgctaatgagcttgatctgctggcgcagaagtattccatagagcagctgaccacttactggctgcagccaggggatgattttgaggaggctattagggtatatgcaaaggtggcacttaggccagattgcaagtacaagatcagcaaacttgtaaatatcaggaattgttgctacatttctgggaacggggccgaggtggagatagatacggaggatagggtggcctttagatgtagcatgataaatatgtggccgggggtgcttggcatggacggggtggttattatgaatgtaaggtttactggccccaattttagcggtacggttttcctggccaataccaaccttatcctacacggtgtaagcttctatgggtttaacaatacctgtgtggaagcctggaccgatgtaagggttcggggctgtgccttttactgctgctggaagggggtggtgtgtcgccccaaaagcagggcttcaattaagaaatgcctctttgaaaggtgtaccttgggtatcctgtctgagggtaactccagggtgcgccacaatgtggcctccgactgtggttgcttcatgctagtgaaaagcgtggctgtgattaagcataacatggtatgtggcaactgcgaggacagggcctctcagatgctgacctgctcggacggcaactgtcacctgctgaagaccattcacgtagccagccactctcgcaaggcctggccagtgtttgagcataacatactgacccgctgttccttgcatttgggtaacaggaggggggtgttcctaccttaccaatgcaatttgagtcacactaagatattgcttgagcccgagagcatgtccaaggtgaacctgaacggggtgtttgacatgaccatgaagatctggaaggtgctgaggtacgatgagacccgcaccaggtgcagaccctgcgagtgtggcggtaaacatattaggaaccagcctgtgatgctggatgtgaccgaggagctgaggcccgatcacttggtgctggcctgcacccgcgctgagtttggctctagcgatgaagatacagattga

SEQ ID NO: 16 - DNA, 1296 bp, synthetic construct
  source 1..1296: mol_type = other DNA
cgttacataacttacggtaaatggcccgcctggctgaccgcccaacgacccccgcccattgacgtcaataatgacgtatgttcccatagtaacgccaatagggactttccattgacgtcaatgggtggagtatttacggtaaactgcccacttggcagtacatcaagtgtatcatatgccaagtacgccccctattgacgtcaatgacggtaaatggcccgcctggcattatgcccagtacatgaccttatgggactttcctacttggcagtacatctacgtattagtcatcgctattaccatggtgatgcggttttggcagtacatcaatgggcgtggatagcggtttgactcacggggatttccaagtctccaccccattgacgtcaatgggagtttgttttggcaccaaaatcaacgggactttccaaaatgtcgtaacaactccgccccattgacgcaaatgggcggtaggcgtgtacggtgggaggtctatataagcagagctcgtttagtgaaccgtcagatcgcctggagacgccatccacgctgttttgacctccatagaagacaccggccgccaccatgactgccctgaccgaaggtgctaagctgtttgagaaggagattccgtacatcaccgagctggaaggggacgtcgaaggaatgaagttcatcatcaagggagaaggaaccggggacgctacgactggaaccattaaggccaagtatatctgtaccactggagatctgccagtgccttgggccacccttgtgtcaaccctctcgtatggagtgcagtgttttgctaagtaccctagccacattaaggacttcttcaaatccgccatgccggaaggttatacccaagagcgcaccatttcttttgagggagatggagtgtacaagacccgcgcgatggtcacctatgagaggggatctatctacaaccgggtgactctgactggagaaaactttaagaaggacgggcatattcttcggaagaatgtcgccttccagtgccctcccagcatcctttacattctccccgacactgtgaacaacggaatccgcgtggagttcaatcaagcctacgacatcgagggggtgacggagaagctggtgaccaagtgtagccagatgaatcggccactggccggttcagcggctgtccacattccgcgctaccatcatatcacttatcacactaagctctccaaagaccgcgatgagaggagagatcacatgtgcctggtggaagtggtcaaggccgtcgatctcgatacctatcagtaa

SEQ ID NO: 17 - DNA, 455 bp, synthetic construct
  source 1..455: mol_type = other DNA
tggcccctccctcgggttaccccacagcctaggccgattcgacctctctccgctggggccctcgctggcgtccctgcaccctgggagcgcgagcggcgcgcgggcggggaagcgcggcccagacccccgggtccgcccggagcagctgcgctgtcggggccaggccgggctcccagtggattcgcgggcacagacgcccaggaccgcgctccccacgtggcggagggactggggacccgggcacccgtcctgccccttcaccttccagctccgcctcctccgcgcggaccccgccccgtcccgacccctcccgggtccccggcccagccccctccgggccctcccagcccctccccttcctttccgcggccccgccctctcctcgcggcgcgagtttcaggcagcgctgcgtcctgctgcgcacgtgggaagccctggccccggccacccccgcg

SEQ ID NO: 18 - DNA, 900 bp, unidentified
  source 1..900: mol_type = genomic DNA
acaccgggactgaaaatgagacatattatctgccacggaggtgttattaccgaagaaatggccgccagtcttttggaccagctgatcgaagaggtactggctgataatcttccacctcctagccattttgaaccacctacccttcacgaactgtatgatttagacgtgacggcccccgaagatcccaacgaggaggcggtttcgcagatttttcccgactctgtaatgttggcggtgcaggaagggattgacttactcacttttccgccggcgcccggttctccggagccgcctcacctttcccggcagcccgagcagccggagcagagagccttgggtccggtttctatgccaaaccttgtaccggaggtgatcgatcttacctgccacgaggctggctttccacccagtgacgacgaggatgaagagggtgaggagtttgtgttagattatgtggagcaccccgggcacggttgcaggtcttgtcattatcaccggaggaatacgggggacccagatattatgtgttcgctttgctatatgaggacctgtggcatgtttgtctacagtcctgtgtctgaacctgagcctgagcccgagccagaaccggagcctgcaagacctacccgccgtcctaaaatggcgcctgctatcctgagacgcccgacatcacctgtgtctagagaatgcaatagtagtacggatagctgtgactccggtccttctaacacacctcctgagatacacccggtggtcccgctgtgccccattaaaccagttgccgtgagagttggtgggcgtcgccaggctgtggaatgtatcgaggacttgcttaacgagcctgggcaacctttggacttgagctgtaaacgccccaggccataaggtgtaaacctgtga

SEQ ID NO: 19 - DNA, 1797 bp, unidentified
  source 1..1797: mol_type = genomic DNA
catggaggcttgggagtgtttggaagatttttctgctgtgcgtaacttgctggaacagagctctaacagtacctcttggttttggaggtttctgtggggctcatcccaggcaaagttagtctgcagaattaaggaggattacaagtgggaatttgaagagcttttgaaatcctgtggtgagctgtttgattctttgaatctgggtcaccaggcgcttttccaagagaaggtcatcaagactttggatttttccacaccggggcgcgctgcggctgctgttgcttttttgagttttataaaggataaatggagcgaagaaacccatctgagcggggggtacctgctggattttctggccatgcatctgtggagagcggttgtgagacacaagaatcgcctgctactgttgtcttccgtccgcccggcgataataccgacggaggagcagcagcagcagcaggaggaagccaggcggcggcggcaggagcagagcccatggaacccgagagccggcctggaccctcgggaatgaatgttgtacaggtggctgaactgtatccagaactgagacgcattttgacaattacagaggatgggcaggggctaaagggggtaaagagggagcggggggcttgtgaggctacagaggaggctaggaatctagcttttagcttaatgaccagacaccgtcctgagtgtattacttttcaacagatcaaggataattgcgctaatgagcttgatctgctggcgcagaagtattccatagagcagctgaccacttactggctgcagccaggggatgattttgaggaggctattagggtatatgcaaaggtggcacttaggccagattgcaagtacaagatcagcaaacttgtaaatatcaggaattgttgctacatttctgggaacggggccgaggtggagatagatacggaggatagggtggcctttagatgtagcatgataaatatgtggccgggggtgcttggcatggacggggtggttattatgaatgtaaggtttactggccccaattttagcggtacggttttcctggccaataccaaccttatcctacacggtgtaagcttctatgggtttaacaatacctgtgtggaagcctggaccgatgtaagggttcggggctgtgccttttactgctgctggaagggggtggtgtgtcgccccaaaagcagggcttcaattaagaaatgcctctttgaaaggtgtaccttgggtatcctgtctgagggtaactccagggtgcgccacaatgtggcctccgactgtggttgcttcatgctagtgaaaagcgtggctgtgattaagcataacatggtatgtggcaactgcgaggacagggcctctcagatgctgacctgctcggacggcaactgtcacctgctgaagaccattcacgtagccagccactctcgcaaggcctggccagtgtttgagcataacatactgacccgctgttccttgcatttgggtaacaggaggggggtgttcctaccttaccaatgcaatttgagtcacactaagatattgcttgagcccgagagcatgtccaaggtgaacctgaacggggtgtttgacatgaccatgaagatctggaaggtgctgaggtacgatgagacccgcaccaggtgcagaccctgcgagtgtggcggtaaacatattaggaaccagcctgtgatgctggatgtgaccgaggagctgaggcccgatcacttggtgctggcctgcacccgcgctgagtttggctctagcgatgaagatacagattga

SEQ ID NO: 20 - DNA, 572 bp, synthetic construct
  source 1..572: mol_type = other DNA
cccctctccctcccccccctaacgttactggccgaagccgcttggaataaggccggtgtgcgtttgtctatatgttattttccaccatattgccgtcttttggcaatgtgagggcccggaaacctggccctgtcttcttgacgagcattcctaggggtctttcccctctcgccaaaggaatgcaaggtctgttgaatgtcgtgaaggaagcagttcctctggaagcttcttgaagacaaacaacgtctgtagcgaccctttgcaggcagcggaaccccccacctggcgacaggtgcctctgcggccaaaagccacgtgtataagatacacctgcaaaggcggcacaaccccagtgccacgttgtgagttggatagttgtggaaagagtcaaatggctctcctcaagcgtattcaacaaggggctgaaggatgcccagaaggtaccccattgtatgggatctgatctggggcctcggtgcacatgctttacatgtgtttagtcgaggttaaaaaaacgtctaggccccccgaaccacggggacgtggttttcctttgaaaaacacgatgataa